European Patent Application EP 4 382 541 A1, published June 12, 2024. Title: 双特异性抗体及其应用. Applicant: 上海恩凯细胞技术有限公司. Application CN. The sequence listing filed with the application follows.

SEQUENCE LISTING (11 sequences)

SEQ ID NO: 1 - protein, 15 aa, synthetic construct
GGGGSGGGGSGGGGS

SEQ ID NO: 2 - protein, 15 aa, synthetic construct
GGGGSGGGGSGGGGS

SEQ ID NO: 3 - protein, 217 aa, synthetic construct
APEFEGGPSVFLFPPKPKDTLMISRTPEVTCVVVDVSQEDPEVQFNWYVDGVEVHNAKTKPREEQFQSTYRVVSVLTVLHQDWLNGKEYKCKVSNKGLPSSIEKTISKAKGQPREPQVYTLPPSQEEMTKNQVSLTCLVKGFYPSDIAVEWESNGQPENNYKTTPPVLDSDGSFFLYSRLTVDKSRWQEGNVFSCSVMHEALHNHYTQKSLSLSLGK

SEQ ID NO: 4 - protein, 616 aa, synthetic construct
QVQLVQSGAEVKKPGESLKVSCKASGYTFTSYYMHWVRQAPGQGLEWMGIINPSGGSTSYAQKFQGRVTMTRDTSTSTVYMELSSLRSEDTAVYYCARGSAYYYDFADYWGQGTLVTVSSGGGGSGGGGSGGGGSSYVLTQPSSVSVAPGQTATISCGGHNIGSKNVHWYQQRPGQSPVLVIYQDNKRPSGIPERFSGSNSGNTATLTISGTQAMDEADYYCQVWDNYSVLFGGGTKLTVLESKYGPPCPPCPAPEFEGGPSVFLFPPKPKDTLMISRTPEVTCVVVDVSQEDPEVQFNWYVDGVEVHNAKTKPREEQFQSTYRVVSVLTVLHQDWLNGKEYKCKVSNKGLPSSIEKTISKAKGQPREPQVYTLPPSQEEMTKNQVSLTCLVKGFYPSDIAVEWESNGQPENNYKTTPPVLDSDGSFFLYSRLTVDKSRWQEGNVFSCSVMHEALHNHYTQKSLSLSLGKGGGGSGGGGSGGGGSQDRHMIRMRQLIDIVDQLKNYVNDLVPEFLPAPEDVETNCEWSAFSCFQKAQLKSANTGNNERIINVSIKKLKRKPPSTNAGRRQKHRLTCPSCDSYEKKPPKEFLERFKSLLQKMIHQHLSSRTHGSEDS

SEQ ID NO: 5 - DNA, 1848 bp, synthetic construct
  source 1..1848: mol_type = other DNA
caagttcaattggttcaatctggtgctgaggttaagaaaccaggtgagtctttgaaggtttcttgtaaggcttctggttatactttcacttcttactatatgcattgggttagacaagctccaggtcaaggtttggagtggatgggtattattaatccatctggtggttctacttcttatgctcaaaagttccaaggtagagttactatgactagagatacttctacttctactgtttatatggagttgtcttctttgagatctgaagatactgctgtttattattgtgctagaggttctgcttattattatgatttcgctgattattggggtcaaggtactttggttactgtctcttctggtggtggtggttctggtggtggtggttctggtggtggtggttcctcttacgtcttgactcaaccatcttctgtctctgttgctccaggtcaaactgctactatttcttgtggtggtcataatattggttctaagaatgttcattggtatcaacaaagaccaggtcaatctccagtcttggtcatctatcaagataacaagagaccatctggtattccagagagattctctggttctaattctggtaatactgctactttgactatttctggtactcaagctatggatgaagctgattactattgtcaagtttgggataattattctgtcttgttcggtggtggtactaagttgactgttttggagtccaaatatggtcccccatgcccaccatgcccagcacctgagttcgaagggggaccatcagtcttcctgtttcccccaaaacccaaggacactctcatgatctcccggacccctgaggtcacgtgcgtggtggtggacgtgagccaggaagaccccgaggtccagttcaactggtacgtggatggcgtggaggtgcataatgccaagacaaagccgcgggaggagcagttccaaagcacgtaccgtgtggtcagcgtcctcaccgtcctgcaccaggactggctgaacggcaaggagtacaagtgcaaggtctccaacaaaggcctcccgtcctccatcgagaaaaccatctccaaagccaaagggcagccccgagagccacaggtgtacaccctgcccccatcccaggaggagatgaccaagaaccaggtcagcctgacctgcctggtcaaaggcttctaccccagcgacatcgccgtggagtgggagagcaatgggcagccggagaacaactacaagaccacgcctcccgtgctggactccgacggctccttcttcctctacagcagactaaccgtggacaagagcaggtggcaggaggggaatgtcttctcatgctccgtgatgcatgaggctctgcacaaccactacacacagaagagcctctccctgtctctgggtaaaggtggtggtggttctggaggtggcggttctggtggtggtggttctcaagatcgccacatgattagaatgcgtcaacttatagatattgttgatcagctgaaaaattatgtgaatgacttggtccctgaatttctgccagctccagaagatgtagagacaaactgtgagtggtcagctttttcctgttttcagaaggcccaactaaagtcagcaaatacaggaaacaatgaaaggataatcaatgtatcaattaaaaagctgaagaggaaaccaccttccacaaatgcagggagaagacagaaacacagactaacatgcccttcatgtgattcttatgagaaaaaaccacccaaagaattcctagaaagattcaaatcacttctccaaaagatgattcatcagcatctgtcctctagaacacacggaagtgaagattcc

SEQ ID NO: 6 - DNA, 1410 bp, synthetic construct
  source 1..1410: mol_type = other DNA
caagttcaattggttcaatctggtgctgaggttaagaaaccaggtgagtctttgaaggtttcttgtaaggcttctggttatactttcacttcttactatatgcattgggttagacaagctccaggtcaaggtttggagtggatgggtattattaatccatctggtggttctacttcttatgctcaaaagttccaaggtagagttactatgactagagatacttctacttctactgtttatatggagttgtcttctttgagatctgaagatactgctgtttattattgtgctagaggttctgcttattattatgatttcgctgattattggggtcaaggtactttggttactgtctcttctggtggtggtggttctggtggtggtggttctggtggtggtggttcctcttacgtcttgactcaaccatcttctgtctctgttgctccaggtcaaactgctactatttcttgtggtggtcataatattggttctaagaatgttcattggtatcaacaaagaccaggtcaatctccagtcttggtcatctatcaagataacaagagaccatctggtattccagagagattctctggttctaattctggtaatactgctactttgactatttctggtactcaagctatggatgaagctgattactattgtcaagtttgggataattattctgtcttgttcggtggtggtactaagttgactgttttggagtccaaatatggtcccccatgcccaccatgcccagcacctgagttcgaagggggaccatcagtcttcctgtttcccccaaaacccaaggacactctcatgatctcccggacccctgaggtcacgtgcgtggtggtggacgtgagccaggaagaccccgaggtccagttcaactggtacgtggatggcgtggaggtgcataatgccaagacaaagccgcgggaggagcagttccaaagcacgtaccgtgtggtcagcgtcctcaccgtcctgcaccaggactggctgaacggcaaggagtacaagtgcaaggtctccaacaaaggcctcccgtcctccatcgagaaaaccatctccaaagccaaagggcagccccgagagccacaggtgtacaccctgcccccatcccaggaggagatgaccaagaaccaggtcagcctgacctgcctggtcaaaggcttctaccccagcgacatcgccgtggagtgggagagcaatgggcagccggagaacaactacaagaccacgcctcccgtgctggactccgacggctccttcttcctctacagcagactaaccgtggacaagagcaggtggcaggaggggaatgtcttctcatgctccgtgatgcatgaggctctgcacaaccactacacacagaagagcctctccctgtctctgggtaaa

SEQ ID NO: 7 - DNA, 441 bp, synthetic construct
  source 1..441: mol_type = other DNA
ggtggtggtggttctggaggtggcggttctggtggtggtggttctcaagatcgccacatgattagaatgcgtcaacttatagatattgttgatcagctgaaaaattatgtgaatgacttggtccctgaatttctgccagctccagaagatgtagagacaaactgtgagtggtcagctttttcctgttttcagaaggcccaactaaagtcagcaaatacaggaaacaatgaaaggataatcaatgtatcaattaaaaagctgaagaggaaaccaccttccacaaatgcagggagaagacagaaacacagactaacatgcccttcatgtgattcttatgagaaaaaaccacccaaagaattcctagaaagattcaaatcacttctccaaaagatgattcatcagcatctgtcctctagaacacacggaagtgaagattcctag

SEQ ID NO: 8 - DNA, 30 bp, synthetic construct
  source 1..30: mol_type = other DNA
ctctcgagaaaagacaagttcaattggttc

SEQ ID NO: 9 - DNA, 26 bp, synthetic construct
  source 1..26: mol_type = other DNA
cggttagtctgctgtagaggaagaag

SEQ ID NO: 10 - DNA, 26 bp, synthetic construct
  source 1..26: mol_type = other DNA
cttcttcctctacagcagactaaccg

SEQ ID NO: 11 - DNA, 30 bp, synthetic construct
  source 1..30: mol_type = other DNA
ttcgcggccgcctaggaatcttcacttccg